European Patent Specification EP 3 690 040 B1, published October 29, 2025. Title: Method for producing protein and method for producing disaccharide. Applicant: Ajinomoto Co., Inc. The sequence listing filed with the application follows.

SEQUENCE LISTING (87 sequences)

SEQ ID NO: 1 - DNA, 1700 bp, Talaromyces cellulolyticus
atgggtagcgtaactagtaccaacggcgagactccccagtccaaactgccggcagactttgtctggggatacgcaacggccaggtgagattactcgctattcatgtgtgtagaagaaacctatttaccgtcttgttttggttctagctaccagatcgaaggagcgtatgacgaagacggccgaggaccttccatctgggatacattcagcaagacacctggaaaagtagaggatggcaccaatggcgacgtggcctgcgactcctaccaccgtacacatgaggatattgcgattctgaagcaatatggtgccaagctgtaccgcttttctctgtcctggtatagctcccttcggcttcttgcgccagaatataactgacagtattgataatcaaggccccgaatcattcctctaggtggccgaaacgaccccatcaaccaaaagggaatagacttttactccaaattcatcgacgatctccacgccgctggaatcgagcccttcgtcaccttgtaccactgggatcttcccgacgagctgttcaagagatacggcggccccctcaacaaggacgaattcgtggctgactatgcgaacttcgcccgcatcgcattccagagctttggacacaaagtcaagcattgggttaccttcaatgaaccatggtgtagctccgtgctcggtttcaatatcggtaagcatgcgccaggacggacgagcgatcgcaagaagaacccggttggtgatggtgtgcgtgagccatggattgctggtcattcccttttggtggctcacggcacggctgttgatatctaccggaaggaatttaagcctacacagggcggagaaattggcattacactcaatggttagatcgaaatattccccaacgcatgacaatcatgcgctaatatgaattcaaggtgactgggccgaaccctgggaccccgaagacccagaagacattgaagcctgcacccgcaaactcgaattcgccatctcctggtttgcagaccccatctaccttggcaaataccccgacagcgtcgtgaaacaaatcggcgaccgtctcccacccttgacacccgatgaagtagccttgatcaagggaagcaacgacttttacggcatgaaccactactgcgcaaactacatccgtcaccgagaaggtgaagcggatccagacgacacagccggaaacttggaccatttgtttgaggataaattcggaaactcgattggacccgagacgaattgtgaatggcttcgccctcatcccttgggattcaggaagttgttgaaatggctttcggatcgttatggttatcccaaaatctatgttacggagaacgggacgagtatcaagggcgagaacgacttgccactagaggaactcctcaatgatgagtttagggtgcagtattaccgggattatgtcggtgccatggctgatgctgctacttttgacggagtcaatgttaagaaatatatggcctggagtttgatggagtaagtcaaaacatcacctattcggaaagacttctgctaatcgctctattagtaacttcgagtggtccgaaggttaccaatccagatttggtgtcacatacgtcgactacaaggacaaccagaaacgtatccccaagaagagtgccctcgtcattggagaattgttcaacaaatacatctcgaaagagtag

SEQ ID NO: 2 - DNA, 45 bp, Artificial Sequence
  primer
cggtacccggggatccacacgagttgctacaacctcaattacctg

SEQ ID NO: 3 - DNA, 43 bp, Artificial Sequence
  primer
ccgatctgaattgacctcggagatgtgttggatgtgattctgc

SEQ ID NO: 4 - DNA, 40 bp, Artificial Sequence
  primer
tcggcgttcacttatcaatcatatcacgctcgctttggcc

SEQ ID NO: 5 - DNA, 42 bp, Artificial Sequence
  primer
cgactctagaggatcgtcataggtggcccgtttaaagacagc

SEQ ID NO: 6 - DNA, 22 bp, Artificial Sequence
  primer
gtcaattcagatcggctgccgc

SEQ ID NO: 7 - DNA, 35 bp, Artificial Sequence
  primer
ataagtgaacgccgagtcagtactatatgtagatg

SEQ ID NO: 8 - DNA, 37 bp, Artificial Sequence
  primer
cggtacccggggatcgtcaattcagatcggctgccgc

SEQ ID NO: 9 - DNA, 50 bp, Artificial Sequence
  primer
cgactctagaggatcataagtgaacgccgagtcagtactatatgtagatg

SEQ ID NO: 10 - DNA, 44 bp, Artificial Sequence
  primer
gattacgccaagcttcgtccttgttgagggggccgccgtatctc

SEQ ID NO: 11 - DNA, 44 bp, Artificial Sequence
  primer
gattacgccaagcttcgaagacggccgaggaccttccatctggg

SEQ ID NO: 12 - DNA, 42 bp, Artificial Sequence
  primer
aagaaggagatatacatgggtagcgtaactagtaccaacggc

SEQ ID NO: 13 - DNA, 73 bp, Artificial Sequence
  primer
gttagcagccggatctcagtggtggtggtggtggtgctctttcgagatgtatttgttgaacaattctccaatg

SEQ ID NO: 14 - DNA, 43 bp, Artificial Sequence
  primer
gtatatctccttcttaaagttaaacaaaattatttctagaggg

SEQ ID NO: 15 - DNA, 23 bp, Artificial Sequence
  primer
gatccggctgctaacaaagcccg

SEQ ID NO: 16 - DNA, 22 bp, Artificial Sequence
  primer
tcttccccatcggtgatgtcgg

SEQ ID NO: 17 - DNA, 21 bp, Artificial Sequence
  primer
gtctggggatacgcaacggcc

SEQ ID NO: 18 - DNA, 24 bp, Artificial Sequence
  primer
ccgaatcattcctctaggtggccg

SEQ ID NO: 19 - DNA, 24 bp, Artificial Sequence
  primer
tatcggtaagcatgcgccaggacg

SEQ ID NO: 20 - DNA, 25 bp, Artificial Sequence
  primer
ttcgccatctcctggtttgcagacc

SEQ ID NO: 21 - DNA, 29 bp, Artificial Sequence
  primer
caggaagttgttgaaatggctttcggatc

SEQ ID NO: 22 - DNA, 1473 bp, Talaromyces cellulolyticus
atgggtagcgtaactagtaccaacggcgagactccccagtccaaactgccggcagactttgtctggggatacgcaacggccagctaccagatcgaaggagcgtatgacgaagacggccgaggaccttccatctgggatacattcagcaagacacctggaaaagtagaggatggcaccaatggcgacgtggcctgcgactcctaccaccgtacacatgaggatattgcgattctgaagcaatatggtgccaagctgtaccgcttttctctgtcctggccccgaatcattcctctaggtggccgaaacgaccccatcaaccaaaagggaatagacttttactccaaattcatcgacgatctccacgccgctggaatcgagcccttcgtcaccttgtaccactgggatcttcccgacgagctgttcaagagatacggcggccccctcaacaaggacgaattcgtggctgactatgcgaacttcgcccgcatcgcattccagagctttggacacaaagtcaagcattgggttaccttcaatgaaccatggtgtagctccgtgctcggtttcaatatcggtaagcatgcgccaggacggacgagcgatcgcaagaagaacccggttggtgatggtgtgcgtgagccatggattgctggtcattcccttttggtggctcacggcacggctgttgatatctaccggaaggaatttaagcctacacagggcggagaaattggcattacactcaatggtgactgggccgaaccctgggaccccgaagacccagaagacattgaagcctgcacccgcaaactcgaattcgccatctcctggtttgcagaccccatctaccttggcaaataccccgacagcgtcgtgaaacaaatcggcgaccgtctcccacccttgacacccgatgaagtagccttgatcaagggaagcaacgacttttacggcatgaaccactactgcgcaaactacatccgtcaccgagaaggtgaagcggatccagacgacacagccggaaacttggaccatttgtttgaggataaattcggaaactcgattggacccgagacgaattgtgaatggcttcgccctcatcccttgggattcaggaagttgttgaaatggctttcggatcgttatggttatcccaaaatctatgttacggagaacgggacgagtatcaagggcgagaacgacttgccactagaggaactcctcaatgatgagtttagggtgcagtattaccgggattatgtcggtgccatggctgatgctgctacttttgacggagtcaatgttaagaaatatatggcctggagtttgatggataacttcgagtggtccgaaggttaccaatccagatttggtgtcacatacgtcgactacaaggacaaccagaaacgtatccccaagaagagtgccctcgtcattggagaattgttcaacaaatacatctcgaaagagtag

SEQ ID NO: 23 - protein, 490 aa, Talaromyces cellulolyticus
MGSVTSTNGETPQSKLPADFVWGYATASYQIEGAYDEDGRGPSIWDTFSKTPGKVEDGTNGDVACDSYHRTHEDIAILKQYGAKLYRFSLSWPRIIPLGGRNDPINQKGIDFYSKFIDDLHAAGIEPFVTLYHWDLPDELFKRYGGPLNKDEFVADYANFARIAFQSFGHKVKHWVTFNEPWCSSVLGFNIGKHAPGRTSDRKKNPVGDGVREPWIAGHSLLVAHGTAVDIYRKEFKPTQGGEIGITLNGDWAEPWDPEDPEDIEACTRKLEFAISWFADPIYLGKYPDSVVKQIGDRLPPLTPDEVALIKGSNDFYGMNHYCANYIRHREGEADPDDTAGNLDHLFEDKFGNSIGPETNCEWLRPHPLGFRKLLKWLSDRYGYPKIYVTENGTSIKGENDLPLEELLNDEFRVQYYRDYVGAMADAATFDGVNVKKYMAWSLMDNFEWSEGYQSRFGVTYVDYKDNQKRIPKKSALVIGELFNKYISKE

SEQ ID NO: 24 - DNA, 40 bp, Artificial Sequence
  primer
cggtacccggggatccccttcttgccagcacactgctccg

SEQ ID NO: 25 - DNA, 40 bp, Artificial Sequence
  primer
agctgcgaggtcaacggctaagcgccagtttggtgaatcc

SEQ ID NO: 26 - DNA, 40 bp, Artificial Sequence
  primer
aactggcgcttagccgttgacctcgcagctggcacgggat

SEQ ID NO: 27 - DNA, 40 bp, Artificial Sequence
  primer
cgactctagaggatccgccaagggatccgtgagatcgcat

SEQ ID NO: 28 - DNA, 43 bp, Artificial Sequence
  primer
acctgactcgaccggctcggagatgtgttggatgtgattctgc

SEQ ID NO: 29 - DNA, 40 bp, Artificial Sequence
  primer
gcttgttgacctcgccaatcatatcacgctcgctttggcc

SEQ ID NO: 30 - DNA, 28 bp, Artificial Sequence
  primer
ccggtcgagtcaggtattcatatcatcc

SEQ ID NO: 31 - DNA, 25 bp, Artificial Sequence
  primer
gcgaggtcaacaagcctcaaaccct

SEQ ID NO: 32 - DNA, 40 bp, Artificial Sequence
  primer
cggtacccggggatcagcgcagaccaatgccagaggagaa

SEQ ID NO: 33 - DNA, 40 bp, Artificial Sequence
  primer
ccgatctgaattgacgcgcgagttgcgcgatgaaatttat

SEQ ID NO: 34 - DNA, 40 bp, Artificial Sequence
  primer
tcggcgttcacttatcttccccaagaccgtaagtcggggc

SEQ ID NO: 35 - DNA, 40 bp, Artificial Sequence
  primer
cgactctagaggatcaaccgtcgatcagaaggagcgcaat

SEQ ID NO: 36 - DNA, 20 bp, Artificial Sequence
  primer
gtcaattcagatcggctgcc

SEQ ID NO: 37 - DNA, 20 bp, Artificial Sequence
  primer
ataagtgaacgccgagtcag

SEQ ID NO: 38 - protein, 813 aa, Talaromyces cellulolyticus
MYSAFLLLLASATPIVSAQSASWSAAYSKATAALSKLSQNDKIGMVTGVGWGKGPCVGNTAAPSGISFPSLCIQDSPLGVRYANPVTAFPAGTNAGMTWDRTLMNQRGAALGAESKGLGVHVQLGPVAGPLGKIAQGGRGWEGFGTDPYLSGVAMIETISGMQSSGTQACAKHYIGNEQELNRESMSSNIDDRTLHELYLWPFADAVRANVASVMCSYNQINGTFSCENEESMTGILKTELGFPGYIMSDWDAQHTTVTSANSGLDMTMPGSDYSDTPSSVLWGQNLANAISSGQVAQSRLDDMVTRILAAWYLVGQDQGFPAVAFNSWTGGQASVNVTSNHNQVARAVARDSIVLLKNTNSTLPLNKPSSIAIIGTDAQTNPSGPNACTDRGCDTGTLAMGWGSGTCQFPYLTDPLTAIKTRAASDGTTITTSISDNGSAGASVAQSAEYAIVFINSDSGEGYITVEGVAGDRNNLDPWHSGNALVQSVAAVNKKTIVVIHSVGPVILETILAQPNVVAVVWAGIPGQESGSALTDILYGSTAPSGKLTYTIAKQASDYGTAVVSGSDNYPEGLFIDYRHFDKSNIEPRYEFGYGLSYTTFGYTNLAIDITVSTGPTTGQIVPGGPSDLFESVGTVTVQVANTGSVAGSEVAQLYIGLPSSAPSSPPKQLRGFDKLSLAAGASGTATFDLTRRDLSYWDVSKQKWVVPSGAFTVYVGASSRDIRLQGTFTPGGSSTTSTITSSKTSTTISTSVTTSSSTTAKTTTTSSTTSSAGPTQTPYGQCGGQGWTGPTVCSSGWTCKVTNQWYSQCLQ

SEQ ID NO: 39 - DNA, 40 bp, Artificial Sequence
  primer
tcgagctcggtaccccgaggtctgtctaaaaaatctagca

SEQ ID NO: 40 - DNA, 40 bp, Artificial Sequence
  primer
ccgatctgaattgactttgatatgttcttctcttgaacct

SEQ ID NO: 41 - DNA, 40 bp, Artificial Sequence
  primer
tcggcgttcacttatggtacgggagatgaacgttgggaat

SEQ ID NO: 42 - DNA, 40 bp, Artificial Sequence
  primer
ctctagaggatcccctgaaagacgagaacgacataaagcg

SEQ ID NO: 43 - DNA, 20 bp, Artificial Sequence
  primer
gtcaattcagatcggctgcc

SEQ ID NO: 44 - DNA, 20 bp, Artificial Sequence
  primer
ataagtgaacgccgagtcag

SEQ ID NO: 45 - DNA, 20 bp, Artificial Sequence
  primer
gtccttttataaccgagcca

SEQ ID NO: 46 - DNA, 20 bp, Artificial Sequence
  primer
ctggaacatacaagtccggc

SEQ ID NO: 47 - DNA, 4509 bp, Talaromyces cellulolyticus
atgtcgagaagaatacggaaccctgattccgcaggctcgagtcaaaccctaagtaattcaccggtaccaatagccgccgaatccggcacggaacctgtgtacctaggtccgtatcgaatagcgaagttttccgtctattcttcgaattttgtatacatgcttaccttggctcaaaggtactcacaaagtccgaagaataaattatagaaccgatgtgaaacggggacagtttggcaaccccttgtactatgtacattgtatggatctcgtctcgactctcgagacgagggtttcgtaccaaccaaagactcaaaacttggggtaactaagcgatcggctgcgtagtactccatactccataaataccccggtgaattcgcctcttgcccatggaatgagcgagaatttacccttggagtcatcgcggtaaatgactcacatatcatgtctgccttcactctcctcaacctttgaaattccggttaatgttaaggcgaggtgtcctctacggaatggctttgtagatttgagataagactacgccgtaacttaagggatccacatactccatattgatagtctcaggaccgagatagtctggagtaaccccgtacccaatcaacgtcctcagactcgccacctggttacaatatttcggtgcttgtgccgatatacctccgttgcgtgagccttgatagccaacaagaaatgattcaaaattaagatttgagaaaatccggagtacgcagtgcctgcagtgtaaaaaataatgtatttacctaatgccaatatgtcgatgccaaagtactactagcaaagacactagatatgcagcaaactcgatgtttaggtacatgtaaccatatcctggggtcaggtacgaacgccatcaattaatctcgtaaactagctgtcacacgacagtatcatttgatagttccaatgttccatgctccccctcaaatgtcactggatgatacgaatttggctgtgacttgaacagatagacggaaaacagtccgatcattatccggagtacgcatgtacgagatagtctggggatcctcggctgccccgattggggttagtgcgggtttccttatcttgatacgccgtctggaggcgcaggtgattgttacggtgtgttccgtgatagataagttagacatccgataataacctatcttctagatagacggcaggtacgtatgtagatagatagatgacacagtcataagacagttttatttaccatacatagtatagtcatttgacaaacacttgatgactatgagcagtaagtccagacaagagcatagactagaaatgatgtgatcatcaataggtacggagtcgtaccacccccggattatcttggctggcttagtcacgcccaaacagacggtgacggatgagacacaagcaaagagcgacattccgaagaattctcgtgacggaaacgagaatgccgccggcgctgatagggggaaattttatcttttccctttctgacattcagtgtttacaatacaatacggaattacggaaccccggttttcgcaaccggtggaattacctaatgggtgacctgaatttattagataacgatgaacaatttgttggatcttccgtagatcgatttggacttgataggtgcttccaaggttgttgctgctcacatggtcgcttgcgttatctgcctacagaatgaggaagatgtattccgcacgtactccggtcgcgacagatatgcgacgattgcaatatgtactacatagttagtacatacaactctagactagactctatattatgtagagtgtaagagaaaaagaaagaagataacggcagggtctatttgattgcgctataatatgcgccgctgtatggttccccagatctgcgtgagatatcacctcatcctatcatcattccaggtcaaagtctcgtcatcatgaattggtattattacccagtacgtaaaccacgtatcgaggcgtatcggtgtattaaagatagagctactgcattggctctagtcctatctttgccccggaatccggcccgtggatgacgatatgatgctgtttgtccttcagctaaacacggacgatctcttacagggtgcggttaattattaaggatataattctaatcaacgactctggctgtgctatattaacaatgtcttctaagtggtcatgatgtgtacgtacttcgtacacatgctacatgcaatcgagtacgtaactccagatctgcgccgtacccgcgatacccgggccatcatgcaaatgtaaccgcttggaacacgcactgcagtgcataaaagccacagcctcgcttcccaatccggtttagacgcgttttgtcttgctgttttgggagcagccagaccccacattccactaacccactctttttcagcgcttattctcgtaagattcgtacgaaaaatacatctgcccacactatccaccagctcggccactcttcggtgagaacgctgccatgagaaaaaaatctgcgactctgcaacagagtgaggcacggctgaaccgagctgattgtcaccctttgcccaatgcccagacagcccagacagcccagacagcccagacagcccagacagcccagacagcccagacagccagtgcttggttaatttttactaagggtaaaaacctaaaaaaaagaaacgaaaaaaaaaaaaaaaaacttttcttttttgccccccaatcacttggccgacagtcaaagggttcccccacacggtactccgtacttgctacgtacactaactaaagaaaaaatctcctgattgagtctgtgtctgtctgtcgctgctaaactcggataaccccccgttcccgatcacccgtcgaaaagagcagcagccatttaacatttttcccctccattcctccttcttggaactttccctccctccctcatccttacatctccctgcgtgcgcgcctgcctgcctacttacactgccactccccagattttctttctcttgtttcttctccagactttctttcctcctccacctcgcctcaccacaccaccaccaccactcaccacgccaacaacaccgcactaccactactgcttcaaagatcgatcaggccattatcaaggaggatcgacgtcttattccatcgaccaccctgttgatcacctcggctggagcgctcgactccctggcttccttccccagcttatttaaacccgtcacccgccaggtctcttcacatgtcaccgtcatcttcgtcagtgggtttttccaatctgctgaacccacagtcagactctgtcgagcctacggataacacatcttcacctgctaccaccactaccaccggcacagactccaactcagacaaggaaatggcgtcctctgtcagtctgctcccaccactcatgaagggtgcccgccccgccgcggaggaagtgcgacaggacctccctcgtccatacaagtgtcctctttgcgatcgtgctttccatcgtctagagcaccaaactcgtcacattcgtactcacaccggcgagaaaccccatgcctgccagtttccaggctgcacgaaacggttcagtcgttcagatgaattgactcgtcactcgcgcattcacaacaaccccaactcgagaagaagtaacaaagctcagcatattgctgcggctgcggcggccggtcaggattcgggtatgcttaacgctgctgcctcgatgatgcctcctccaagcaaacccattactcgctcggctccagtgtctcaggtcggatctccggatgtgtctcctccgcactcttacaccaactacacctcgcatttgcgggcgggtctgggtccttattcacgcaacagcgaccgtgcttcatctggtatggatattaatttgctcgcgactgctgcttcacaagtcgagcgcgatcactacggaggctcgtctcgtcattaccctttcagctctcgatactcgggtactcctggacgtctaccgtcgctttccgcctatgccatttctcagagcatgagccggtcgcattctcacgaggatgaggacaactacggacatcaccgggttaagcgctctcgtcctaactcaccaaactcgactgcgccatcctcgcctacattctctcacgattcattgtcgcctacccccgatcacactcctcttgcaaccccagcacactcgcctcgtttgcgtccttatggagccgcagatttgcaattaccttccatccgtcatttgtcgttacaccacactcccgcactcgcaccaatggagcctcaagccgagggacctaatgtttacaaccccggtcagcaccacggtggacccagcatcacggacatcatgagcaggcccgacggcacccagcgtaagcttcctgttccgcaagtacccaaaatcccggtgcaggacatgttggcaccgaacggatattcctccaacactccgtccgtcaacggttccgtgatggagttataa

SEQ ID NO: 48 - DNA, 2442 bp, Talaromyces cellulolyticus
atgtattccgcatttcttttgctgctggcttcggccacgcctatagtcagcgcccagtcagcttcttggtccgcagcctacagtaaagccacggctgctttgagcaaactctctcaaaatgacaaaattggtatggtgacaggcgtgggatgggggaaaggtccatgtgttggaaacactgccgcgccatctggaatctcgtttccatcactctgtattcaagatagtcccctaggcgttcgttatgcgaaccccgtcacagcgtttccggcaggcacgaatgctggaatgacctgggatcggacgttgatgaaccagagaggtgccgctcttggtgcagaatccaaggggctaggtgtccatgttcagttagggcctgtggcaggtcccctaggaaagatcgcgcagggtggtcgtggttgggaaggatttggaacggatccatacctcagtggtgttgctatgattgagactatttcaggtatgcagagttcgggtactcaggcatgcgcgaagcactatattggcaacgagcaagagctaaacagggaatcgatgagttctaatattgatgatcgtactttgcacgagctttacctgtggccctttgccgatgccgtccgtgccaatgttgccagtgtgatgtgctcctacaaccaaatcaatggaacattttcctgtgagaatgaagaatcgatgacaggtattctgaagacagagctcggctttccaggatacataatgtctgactgggatgcacagcacaccacagttactagtgctaactctggacttgatatgacgatgccaggtagtgattatagtgatacgccgagtagtgtcctttggggtcaaaatctggccaatgccatctcaagtggccaagttgcccagtcgcgtctcgacgatatggtgactcgaattttggctgcttggtatttggttgggcaggatcaaggcttccctgcggtggcctttaactcttggaccggtgggcaagcaagtgttaatgtcacatcaaaccacaaccaagttgcccgtgcagtcgctcgcgattctatcgttttgcttaaaaataccaatagcacgcttccgttgaacaaaccatcgagcattgctattattggcactgacgcccagacaaacccttccgggccaaacgcttgtactgatcgtggttgtgatactggaactttggctatgggttggggtagtggaacttgccaatttccatatctcacagatcctctaacagctattaaaactcgagctgccagcgacgggactacgatcacgacgagcattagtgacaatggcagtgcgggagcctcagttgctcaaagcgccgagtatgcaatcgttttcatcaattcagactctggcgaagggtacataacagtcgaaggcgtcgctggtgaccgcaacaatctcgacccatggcacagtggcaatgcattagtgcaatccgtcgccgcagtcaacaagaagacgattgtcgtcattcatagcgtcgggccggtcattcttgaaaccatattggcgcaacctaacgttgtggccgtagtatgggctggcataccaggacaagagagcggctcagccctcaccgatattctctatgggagtacagctcccagtggaaagctaacgtacacgattgccaaacaggcttccgattacggcactgcagtcgtcagtggtagcgacaattatccagagggacttttcattgattaccgacacttcgacaaaagcaatattgaacctcgatatgaattcggctatggactgtcatatacaacctttggttacacgaatttggcaattgatattacggtttcgacgggcccaactactggtcaaatagttcctggtggaccttctgatctttttgagtctgttggaaccgttacggtacaggtcgcaaacacaggcagcgttgcaggctcagaagttgcacaactctatattgggctgccatcgtcagcaccgtcatcaccaccaaaacagttgcgtgggtttgataagctttctctcgctgctggcgctagcgggaccgcaacgttcgatttgacacgaagagatttgagttactgggatgtatcaaagcagaagtgggtggttccaagcggagcatttaccgtatatgttggggcatcgagtagggatattaggttgcaggggacatttacgcccggaggtagctcgaccacttcgactataacttcctctaagacttctactactatcagcacttctgttaccaccagtagcagtacgacagctaaaaccaccacaactagctcgaccacgtcatctgccgggccaacacagaccccgtatggacagtgtggtggacagggttggaccggccctacagtgtgttcatctggctggacttgcaaggtaacgaatcaatggtattctcaatgcctacaatag

SEQ ID NO: 49 - DNA, 1354 bp, Talaromyces cellulolyticus
ctcgtgaaagctgccctcacaatgatcgtcaagatgacgtagtttgactgggtcgttcctggataagggttagggtaaatagggctcaaagtaccacgtgagtgtggaaagataagccctaaccctaaggtcgtgtcggacaaaaattatcacttgaccaaaattggagatccccttaatggagctttttggtaatggtttgtatagggttatgtgacgtccgtatcacatgatttttatcccaacaggtcgatccccctcttatagttaatggacaacatataagtacgtagcatcttagatagttcgtcagcgtcaactgaccaaagtccccgtgtttcattttaatttgtcagactgcaagagtctcgaaacataaaaagatcgaaagttttgccttattaggctatgagcatgaatgtcggaacaatgccgttgaggctattcccaatttcggaaatatgtatcttcattgctgtcgacttgacgacagtcgataaaaggctcatccggatagataagccagatcactcattatgccaatttctccggtgtctgaaaacgtatactacatacgtaactgatcttcgtggttgaaagagtgtttcttctcattctcatctgccgatgccgagccaattggaacaaaccccgcatatggtcctgaatatcaatcgcggagatgcggagagtgagggagcaacacaattttaaattagtcagttttctcatgttctccgcaatcttgcaggcttgggtctggtaggtttatctctctcttttcacaacaaggttgggccattgtcagcttagcaagcgcgcagcaaagggtgtcggtcaatgttcatgtcctccgcggtcactacaaaacagcacgtggggaatgttgctttccctgttgatgttcatgtgttgtcattcccggcaaatcgactccaattaatatggtaggctcctgcataatgcaagtccttgagatgcagcttccggcagatggacgtatagatcagggactttgaggggctaaaacacttacccgagctaaaacataccataatttcgtttaatgactttcgtctggatggcagaggctgaaggtcgattatgagtgaaattggtatgaagccacatacgccgatactgtaacgctgtgccttcatccgccttctatcgcgccccgacattccgcggtaccgcgattatgaagaaaaacactcgtaatgatgaggagatagttcttagctcttattatttttgtctagctatggaatgcaagtttagcactatataatggtggtgtttcccttgaagaattaggcactatcaaccgcaacagtcagaagcaatcgacaca

SEQ ID NO: 50 - DNA, 1100 bp, Talaromyces cellulolyticus
tgctatgcagttgatgctactgtgttctaaaataattgatagggttagggtcgggtataaggcgatgcaatgtatcaattatcacgagaaataatgcagaaaaacacaattccccgtatctgttgattcttaaacaatctgatcaccaatttgtagaaagaaacgattataaggtgccatggtaatgctggagtttacacaggatactacttgttctgttcattacaatgaaccgtaattgcattctgttttgaccactcaacaaatcctacacaaaagtaagtggacttcagtgctcgctctacgcaagtaaatacttggcatatatggcctcgtatattcttacaatgaggtaaattccgatagattactgcccaactagtcaatcttaaatccttaagagatacagggggaggcggaagtacctgaaaccacgtaataagacgttcagggtcatgtgaatgtatgtagtatccatgtccaatacaattgataatagtatccagtattatatctcattcaggtaagcgccacgcgattcttcagatctacttaactgccgactcgccaaacgaaacaacgtttattcgtgaccccagaaaatcaccgcggagttgcggaggaccagtttgtacaatgcaccgaaccaagcgttggtcatttttctggaaatgggccaaacgttagaagtgattggtcagagctacatctgaaggtgaagcaatttccggtatgcatacatgacagcaagcttacctaccaagaccaagttattccccagcatttgccccatacttggctttaatattgtgggatagcaaacaatatccacaacactgatgataactaaactacaaatctgacgttacttcagactactcacgtgtcaaaagcagttagcgaggatcaagtcttttagtctggtcattaacaaacgcaatttcgcaacccgataatccgcgatgataatatagcgactccaaggtcgtatttatattcaatcaattccccccaatttggaatggatttttggaatcatcgcatgccaggacaatcagtgaaacagtgacaaagtgaagcttcttgatcatttagcaact

SEQ ID NO: 51 - protein, 26 aa, Talaromyces cellulolyticus
MSALNSFNMYKSALILGSLLATAGAQ

SEQ ID NO: 52 - DNA, 24 bp, Artificial Sequence
  primer
cgtctcgggtccaatcgagtttcc

SEQ ID NO: 53 - DNA, 51 bp, Artificial Sequence
  primer
attggacccgagacgaattgtgaatttcttcgccctcatcccttgggattc

SEQ ID NO: 54 - DNA, 37 bp, Artificial Sequence
  primer
gaagttactaatagagcgattagcagaagtctttccg

SEQ ID NO: 55 - DNA, 51 bp, Artificial Sequence
  primer
tctattagtaacttcgagttttccgaaggttaccaatccagatttggtgtc

SEQ ID NO: 56 - DNA, 45 bp, Artificial Sequence; identical to SEQ ID NO: 2
  primer

SEQ ID NO: 57 - DNA, 42 bp, Artificial Sequence; identical to SEQ ID NO: 5
  primer

SEQ ID NO: 58 - DNA, 36 bp, Artificial Sequence
  primer
ggttgagtgttgttcgagagtgaacggcagagggtg

SEQ ID NO: 59 - DNA, 25 bp, Artificial Sequence
  primer
caatcatatcacgctcgctttggcc

SEQ ID NO: 60 - DNA, 26 bp, Artificial Sequence
  primer
gaacaacactcaaccctatctcggtc

SEQ ID NO: 61 - DNA, 28 bp, Artificial Sequence
  primer
aggctttacactttatgcttccggctcg

SEQ ID NO: 62 - DNA, 1589 bp, Talaromyces cellulolyticus
atgaagggcgtcctcagcctttcgctgctgccgttgttgacggttgcgtcaccggtgatgccgcgcaccatccacaacgacgctgctcccattctctcttcgtccaacgccgttgaggtcccagattcatatatcattgtctttaaagaccatgtagattctgcttctgccgcagcccatcataactgggtgcaagacattcacagccaacacaccgagctccgaaagcggtctcaattcccattcgctgacaatgcctttgccggtctcaaacacacttttgacattgccggcagcttccttggttactcaggacacttcgaagagaatgtcattgaggccattcgccgacaccccgatgtgagttatccgcacgtgccctactcctaaggcaatgactaatacgcatctccacctataggttgattacatcgagaaggattctcttgtccacaccatggaagatcccgcccttgagaagaacgccccatggggtttggctcgtatttcgcaccgtgagagcttgagcttcggaagcttcaacaagtacttgtacgctgccgacggcggtgaaggtgttgacgtttatgtcattgacactggtaccaacatcgaccacgtcgacttcgagggtcgtgcttcctggggcaagaccatccccactgacgatgaggatgttgatggcaatggtcacggtactcactgctccggaactattgcgggcaagaagtacggtgttgccaagaaggccaatgtctacgctgtcaaggtcttgaagtctaacggttctggaaccatgtccgatgtcgttcagggtgtcgaatgggctgctactcagcacatcaagaaggtcaaggacgccaaggccggaaaagccaagggcttcaagggtagcgctgcgaacatgagtctcggtggtggcaagtccgtcactcttgacaaggctgtcaatgctgctgttgatgctggtatccacttcgctgtcgctgctggcaacgacaacgccgactcctgcaactactcccctgccgccgctgagaaggccgtcaccgtcggagcctcgaccttggccgatgagcgtgcttacttctccaactacggcaagtgcaacgacatctttgctcctggtctgaacattctctctacctggatcggcagcaagtacgccgtcaacaccatctccggtacctccatggcttctcctcacattgctggtcttttggcctacttcctctctctccagcctgccagtgactccgccttcgctgttgccgagattactcccaagaagttgaaggagaacctcattgctattggtacccagggcgctcttactgatgttccctctgacaccactaacgtaagttgactctgttagtctttcaatgcattatcaactaacaactgtgtcatagattctcgcctggaacggtggtggctcagccaactacaccgacatcattgcccaaggtggttacaagaccaagacactcagcaacgaagttgacgaattgatcaacaagttggaggtcgtgaacgaggaactcggtgccatctacagccacatcaaggatgccattgccgcataa

SEQ ID NO: 63 - DNA, 40 bp, Artificial Sequence
  primer
cggtacccggggatcttggggcacagagacaacagggtca

SEQ ID NO: 64 - DNA, 40 bp, Artificial Sequence
  primer
agatagggttgagtgagatagcgtgagcacactgagcagg

SEQ ID NO: 65 - DNA, 40 bp, Artificial Sequence
  primer
aaagtgtaaagcctgcaacacgctacctcttccacagtag

SEQ ID NO: 66 - DNA, 40 bp, Artificial Sequence
  primer
cgactctagaggatcgagctgattgagcatgctaacgcag

SEQ ID NO: 67 - DNA, 21 bp, Artificial Sequence
  primer
cactcaaccctatctcggtct

SEQ ID NO: 68 - DNA, 24 bp, Artificial Sequence
  primer
caggctttacactttatgcttccg

SEQ ID NO: 69 - protein, 490 aa, Talaromyces cellulolyticus
MKGVLSLSLLPLLTVASPVMPRTIHNDAAPILSSSNAVEVPDSYIIVFKDHVDSASAAAHHNWVQDIHSQHTELRKRSQFPFADNAFAGLKHTFDIAGSFLGYSGHFEENVIEAIRRHPDVDYIEKDSLVHTMEDPALEKNAPWGLARISHRESLSFGSFNKYLYAADGGEGVDVYVIDTGTNIDHVDFEGRASWGKTIPTDDEDVDGNGHGTHCSGTIAGKKYGVAKKANVYAVKVLKSNGSGTMSDVVQGVEWAATQHIKKVKDAKAGKAKGFKGSAANMSLGGGKSVTLDKAVNAAVDAGIHFAVAAGNDNADSCNYSPAAAEKAVTVGASTLADERAYFSNYGKCNDIFAPGLNILSTWIGSKYAVNTISGTSMASPHIAGLLAYFLSLQPASDSAFAVAEITPKKLKENLIAIGTQGALTDVPSDTTNILAWNGGGSANYTDIIAQGGYKTKTLSNEVDELINKLEVVNEELGAIYSHIKDAIAA

SEQ ID NO: 70 - DNA, 78 bp, Talaromyces cellulolyticus
atgtctgccttgaactctttcaatatgtacaagagcgccctcatcttgggctccttgctggcaacagctggtgctcag

SEQ ID NO: 71 - DNA, 1827 bp, Talaromyces cellulolyticus
aagtgggtcaccttcatctctctcctcttcttgttctccagcgcctacagccgtggtgttttccgtcgtgacgcacacaagtccgaagtggcccatcgcttcaaagacctcggtgaggaaaacttcaaggctctcgtcttgattgccttcgctcagtacttgcaacagtgccctttcgaggaccacgtgaagctggtcaacgaagttaccgaattcgccaaaacctgcgttgctgacgagtctgccgaaaactgcgataagtctctgcataccttgttcggcgacaagctctgtactgtcgctaccctccgtgagacctacggagaaatggccgattgttgcgccaagcaggagcctgagcgtaatgagtgctttctgcagcacaaggacgacaaccccaatttgcctcggcttgttcgtcctgaggttgacgtcatgtgtaccgccttccacgataacgaggaaaccttcctcaagaagtacctctacgagatcgcaagacgccatccctacttctacgctcctgaattgctgttctttgccaagcgttacaaggcagcattcactgagtgttgtcaagccgctgacaaggccgcctgcttgctccccaagttggatgaactccgcgatgagggtaaggcctctagcgccaaacagcgccttaagtgcgcctctttgcagaagttcggtgagagagccttcaaagcctgggctgttgctcgtctatcccaacgtttccctaaagccgagtttgctgaagtttccaaactcgtcactgacctgacaaaggtccatactgagtgctgccacggtgacttgttggagtgtgctgatgatcgtgccgatttggcaaagtacatctgcgagaaccaggacagcatctcctccaagttgaaggagtgctgcgaaaagcccttgctcgagaagtcccactgcattgcggaggtcgagaacgacgaaatgcctgccgacttgccttctttggctgctgacttcgtcgaaagcaaggatgtctgcaagaactacgctgaagccaaagacgtgttcttgggcatgttcttgtacgagtatgctcgtcgccaccctgactactccgtggttcttctcctccgtctcgccaagacatacgagacgactttggagaagtgctgtgccgctgccgaccctcacgagtgctatgccaaggtcttcgacgaattcaagcccttagtcgaagaacctcagaacttaatcaagcagaattgtgagctattcgagcaactcggtgagtacaagttccagaacgcgttactggtccggtacaccaagaaggttccccaagtctccactcctaccttggttgaggtctctcgtaacttgggtaaggttggaagcaagtgctgtaagcaccccgaagccaagcgtatgccttgcgctgaagactacctgtcggtcgtcttgaaccaattgtgcgtcttgcacgagaagactcccgttagcgatcgtgttaccaagtgttgtaccgaaagcttggttaaccgtcgtccctgcttctccgctttggaagtcgatgagacttacgttcctaaggagttcaacgccgaaaccttcacctttcacgctgatatctgcactctgtcagagaaagagcgtcagatcaagaagcaaaccgcactcgttgagcttgtcaagcacaaacccaaagccaccaaggaacagctcaaagccgtcatggacgatttcgctgccttcgtcgagaaatgctgcaaagccgacgacaaggagacgtgcttcgcggaagagggcaagaagttggtcgccgctagtcaagctgctcttggtttgtag

SEQ ID NO: 72 - DNA, 497 bp, Talaromyces cellulolyticus
atcagctttgagtgcagcaaaaatgcttccgactgtcttcttatattgatatcatatttttcaattcactttgtctcaagtttcaatatatcgagaaaatagtatcaaagatgaactgtaataattccgatatacctatacaggtttatagtaaattactctatttcataatgcgtccatccgagaagtctggcggccttatcagtagtccaaaacgcctggtttttagacatgtcacctctaatctccgcttgaggaaaatgcgtccgagcaagttctttcgacggggtgtcttgggtcgtagttggagatatgatatttattacttcgaatcctttgatattctcactcttttcaaccgccaaaaggcaagctcttgccactgcgcgaggattaacccatccccagagttgtcgaaccccagattcataccatttatcgtggtgtctttttctaacatctctcaatggggcaacctcatgtattctcaaacaagc

SEQ ID NO: 73 - DNA, 2858 bp, Talaromyces cellulolyticus
gtcaattcagatcggctgccgcctgcgccccaggtgacgtcgatgaaagctgggcctaggtcgtgcatgcggtccatacggtcgtataagttctggacaccttgggcggtctttggggggaagtattcgaaggaaattccaggtcggccggtggccgcctgttcttggagcttttgcccgacatgcatgttgataggtcggtcaattgtctgctttttcaatatcttctcggtatgatgtagcttgcagaacccaagttatgtagttcaattgcaaaatcaagtctgatcaagaccgaaactcaatcccggagcactgaggttcgcactaattgatcaagggtacaagaatgaggggcacaatgaaagcagtcttgaaaatgacaggcagagaaattgaaagaaaggagaagagaggacctccgggacaggagaaatgaaagcaacaaaaccccgaacaagctggagagaagttaaagggagcagcttggtcaccggcaatggatgctcatcataaaaaaggaccctaaacccgttatcggagtccggagaaatgacgctaattcggatttggaagtccccgccaatcgtgggaaattctcgaagcagacaatttgctcgtgacaatcagccagcaatgagagggagactgaaaaatatgtatttacactcaaagaatccgatactgctattaggatcagtgtttttcttataagcaaatgagcgttggacgtggaaaatgaggaatcctcagtccctatactcggtcagcgacggaggggtgcgtgatcggccaatcacagcctattattttatcaacatctgattggctacttccgataagagcgaaatatgcccctccttgcaatttttaccatcaacgctaacagcaacactcaacaaaccattcaatcttgatactcgctcccattagtcaccacgcaggacaacacaacacgacatcgcatctcagctttgaccattcccgccgcaagcgattcgctgtcacaaacgccagataccccaacatggctgcccctccctccgccgatcaggactacaagaccaatctgttgtctttgctgatagccaacgatgcgctcgcatttggcacgttcacattgaaatctggtcgccagtcgccgtattttttgacctcgagtcgtctttatactgcgcctctgctgcgccaggtgtcggccgcgttcgcgaataccatctcgtccccgccttttgtgaatatagctgcagatggcagcattaccccgaactttgacattgtttttgggtatgttaccctattattcgtgcgcctgatatgcgtgtactgatttacttcaaatagccccgcctacaaaggaatccccgaatgcgtcggtgttgtcaacgagctcgctacccgggatgcgctcgccggtaccaagacatgggacaacatcagctactccttcaaccgcaaagaagccaaagaccacggcgaagggggtaacatcgtcggtgcgcctctcaagggaaaacgtgttttgatcgttgacgacgtcatcaccgctggtaccgcgctgcgtgaagctgtcggcattattcaaaaggaaggcggaaccgttgccggtgttgtgttgctgttcgatcgtcaggaacgggtcagtgatacggagcagaagagtgccattggagccgcggagagggaccttggaggcgatattcctatccgtgcggtgttggtattccaggatttgattgataagcttggagataagattggtcaggaggaggtgcgcaggttggaagagtaccggaacacgtacaaggctcaataaatggctgctgtgggatgaaatgggtatattaacgatttatgctaaaaatggctgggtggaatactgcgaaataaatataaatcagcttgaaggatgtatttttagcgcaaagtgatagaattttctatgtaaatagtttgtacaataggattactactttatatgcgttatgcgtatacatttctaaagtgtaaccagtttagctgggagtacaattttaacactcttccatcaatcaggttccagatcagttttctatctacaatcatgactccccagtctctactcctttcaagaatgacgcgttatgttccaagctcccctggttgatggcggtaacccgatatattctagccaggtcaggtcctagtgtgaggactaacacaggcacgtccagtatcgtagcaaatagaatatcagcatatataagtcccctttcccggaccttgctcgagtcagtgactagcaggtacgtacgtacccatcagactatctactatctactatgtacggagtatatagtcggtacttgacgcaaggcgagtctgatagagggacaatatgcagttctgtagccaatcaatcgcggatggcagaccctcgatcgtcattgtggatctttagcttccttatgggcggggcggtggttatttcagagccatttagccaatcatacatcgtagtccgaaagtctaggattatataggctagaccaatctactgtcaaccggtaaagcgggtctctagtctttatcccgacctcctctctttctctttctccgattcgaatgtgacacatacatctgatcaattgataagaatacggattgccgtgtacgtgggctgacagagctgagataaaatatcctggatgtgatatgtggcgcatccagtaccgacactgtgacaggatccgtgtactacaattcattcatcgatcgttggctaggcaaaaagtaggcaaggtttgcagatcgatatcccggtacctggctaaaatcgagacccatctacatatagtactgactcggcgttcacttat

SEQ ID NO: 74 - DNA, 40 bp, Artificial Sequence; identical to SEQ ID NO: 32
  primer

SEQ ID NO: 75 - DNA, 25 bp, Artificial Sequence
  primer
gcgcgagttgcgcgatgaaatttat

SEQ ID NO: 76 - DNA, 40 bp, Artificial Sequence
  primer
tcgcgcaactcgcgctgctatgcagttgatgctactgtgt

SEQ ID NO: 77 - DNA, 30 bp, Artificial Sequence
  primer
agttgctaaatgatcaagaagcttcacttt

SEQ ID NO: 78 - DNA, 45 bp, Artificial Sequence
  primer
acagctggtgctcagaagtgggtcaccttcatctctctcctcttc

SEQ ID NO: 79 - DNA, 25 bp, Artificial Sequence
  primer
ctgagcaccagctgttgccagcaag

SEQ ID NO: 80 - DNA, 25 bp, Artificial Sequence
  primer
tagatcagctttgagtgcagcaaaa

SEQ ID NO: 81 - DNA, 27 bp, Artificial Sequence
  primer
gcttgtttgagaatacatgaggttgcc

SEQ ID NO: 82 - DNA, 40 bp, Artificial Sequence
  primer
tattctcaaacaagcgtcaattcagatcggctgccgcctg

SEQ ID NO: 83 - DNA, 25 bp, Artificial Sequence
  primer
ataagtgaacgccgagtcagtacta

SEQ ID NO: 84 - DNA, 40 bp, Artificial Sequence
  primer
tcggcgttcacttatcctctttctcgccctttcttctcaa

SEQ ID NO: 85 - DNA, 40 bp, Artificial Sequence; identical to SEQ ID NO: 35
  primer

SEQ ID NO: 86 - DNA, 40 bp, Artificial Sequence
  primer
acagctggtgctcagaagtgggtcaccttcatctctctcc

SEQ ID NO: 87 - DNA, 40 bp, Artificial Sequence
  primer
ctcaaagctgatctacaaaccaagagcagcttgactagcg